European Patent Application EP 4 130 262 A1, published February 8, 2023. Title: QPT GENE ENGINEERED PLANT CELL AND USING METHOD OF THE SAME. Applicant: KT&G CORPORATION. The sequence listing filed with the application follows.

SEQUENCE LISTING (32 sequences)

SEQ ID NO: 1 - DNA, 25 bp, Artificial
  Foward primer sequence of F_Q1s
aataagcttggccaaattttaggac

SEQ ID NO: 2 - DNA, 29 bp, Artificial
  reverse primer sequence of R_Q1s
caactttttacattgtgtcaaattccatg

SEQ ID NO: 3 - DNA, 27 bp, Artificial
  forward primer sequence of F_Q1t
aggcatatgttaattgttcgcaaaatc

SEQ ID NO: 4 - DNA, 23 bp, Artificial
  reverse primer sequence of R_Q1t
caccaaaacatgaaagcaaagct

SEQ ID NO: 5 - DNA, 24 bp, Artificial
  forward primer sequence of F_Q2s
gtgctattgcctgttaactctcac

SEQ ID NO: 6 - DNA, 28 bp, Artificial
  reverse primer sequence of R_Q2s
gagcagacacagaaattatttagtgact

SEQ ID NO: 7 - DNA, 25 bp, Artificial
  forward primer sequence of F_Q2t
ggagtgctattgacagttaactcac

SEQ ID NO: 8 - DNA, 26 bp, Artificial
  reverse primer sequence of R_Q2t
agcttcagatacaccaaacttgtaaa

SEQ ID NO: 9 - DNA, 21 bp, Artificial
  nucleotide sequence of sg1
tgtttagagctattcctttca

SEQ ID NO: 10 - DNA, 20 bp, Artificial
  nucleotide sequence of sg2
tgtgtaaaattgcaggttgg

SEQ ID NO: 11 - DNA, 22 bp, Artificial
  nucleotide sequence of sg3
aatacaagagtggagtcattag

SEQ ID NO: 12 - DNA, 23 bp, Artificial
  nucleotide sequence of sg4
ccaaggtctctttaagaagaaaa

SEQ ID NO: 13 - DNA, 22 bp, Artificial
  nucleotide sequence of sg5
gccaccaagaatacaagagtgg

SEQ ID NO: 14 - DNA, 22 bp, Artificial
  nucleotide sequence of sg6
ccaagaatacaagagtggagtc

SEQ ID NO: 15 - DNA, 26 bp, Artificial
  nucleotide sequence of sg7
gcaaaggaagacgggatcatagcagg

SEQ ID NO: 16 - DNA, 25 bp, Artificial
  nucleotide sequence of sg8
gcacttgctgagatgatattcgcgg

SEQ ID NO: 17 - DNA, 23 bp, Artificial
  nucleotide sequence of sg9
acaacattgttatagctgagagg

SEQ ID NO: 18 - DNA, 23 bp, Artificial
  nucleotide sequence of sg10
atatctgctgctggaggtgtcgg

SEQ ID NO: 19 - DNA, 23 bp, Artificial
  nucleotide sequence of sg11
gatcaatgggaggtttgatacgg

SEQ ID NO: 20 - DNA, 13082 bp, Artificial
  V2k_GE
gtttacccgccaatatatcctgtcaaacactgatagtttaaactgaaggcgggaaacgacaatctgatcatgagcggagaattaagggagtcacgttatgacccccgccgatgacgcgggacaagccgttttacgtttggaactgacagaaccgcaacgttgaaggagccactcagccgcgggtttctggagtttaatgagctaagcacatacgtcagaaaccattattgcgcgttcaaaagtcgcctaaggtcactatcagctagcaaatatttcttgtcaaaaatgctccactgacgttccataaattcccctcggtatccaattagagtctcatattcactctcaatccaaataatctgcaccggatctggatcgtttcgcatgattgaacaagatggattgcacgcaggttctccggccgcttgggtggagaggctattcggctatgactgggcacaacagacaatcggctgctctgatgccgccgtgttccggctgtcagcgcaggggcgcccggttctttttgtcaagaccgacctgtccggtgccctgaatgaactgcaggacgaggcagcgcggctatcgtggctggccacgacgggcgttccttgcgcagctgtgctcgacgttgtcactgaagcgggaagggactggctgctattgggcgaagtgccggggcaggatctcctgtcatctcaccttgctcctgccgagaaagtatccatcatggctgatgcaatgcggcggctgcatacgcttgatccggctacctgcccattcgaccaccaagcgaaacatcgcatcgagcgagcacgtactcggatggaagccggtcttgtcgatcaggatgatctggacgaagagcatcaggggctcgcgccagccgaactgttcgccaggctcaaggcgcgcatgcccgacggcgatgatctcgtcgtgacccatggcgatgcctgcttgccgaatatcatggtggaaaatggccgcttttctggattcatcgactgtggccggctgggtgtggcggaccgctatcaggacatagcgttggctacccgtgatattgctgaagagcttggcggcgaatgggctgaccgcttcctcgtgctttacggtatcgccgctcccgattcgcagcgcatcgccttctatcgccttcttgacgagttcttctgagcgggactctggggttcgaaatgaccgaccaagcgacgcccaacctgccatcacgagatttcgattccaccgccgccttctatgaaaggttgggcttcggaatcgttttccgggacgccggctggatgatcctccagcgcggggatctcatgctggagttcttcgcccacgggatctctgcggaacaggcggtcgaaggtgccgatatcattacgacagcaacggccgacaagcacaacgccacgatcctgagcgacaatatgatcgggcccggcgtccacatcaacggcgtcggcggcgactgcccaggcaagaccgagatgcaccgcgatatcttgctgcgttcggatattttcgtggagttcccgccacagacccggatgatccccgatcgttcaaacatttggcaataaagtttcttaagattgaatcctgttgccggtcttgcgatgattatcatataatttctgttgaattacgttaagcatgtaataattaacatgtaatgcatgacgttatttatgagatgggtttttatgattagagtcccgcaattatacatttaatacgcgatagaaaacaaaatatagcgcgcaaactaggataaattatcgcgcgcggtgtcatctatgttactagatcgggcctcctgtcaatgctggcggcggctctggtggtggttctggtggcggctctgagggtggtggctctgagggtggcggttctgagggtggcggctctgagggaggcggttccggtggtggctctggttccggtgattttgattatgaaaagatggcaaacgctaataagggggctatgaccgaaaatgccgatgaaaacgcgctacagtctgacgctaaaggcaaacttgattctgtcgctactgattacggtgctgctatcgatggtttcattggtgacgtttccggccttgctaatggtaatggtgctactggtgattttgctggctctaattcccaaatggctcaagtcggtgacggtgataattcacctttaatgaataatttccgtcaatatttaccttccctccctcaatcggttgaatgtcgcccttttgtctttggcccaatacgcaaaccgcctctccccgcgcgttggccgattcattaatgcagctggcacgacaggtttcccgactggaaagcgggcagtgagcgcaacgcaattaatgtgagttagctcactcattaggcaccccaggctttacactttatgcttccggctcgtatgttgtgtggaattgtgagcggataacaatttcacacaggaaacagctatgaccatgattacgccaagcttcacgtgaacatggtggagcacgacacacttgtctactccaaaaatatcaaagatacagtctcagaagaccaaagggcaattgagacttttcaacaaagggtaatatccggaaacctcctcggattccattgcccagctatctgtcactttattgtgaagatagtggaaaaggaaggtggctcctacaaatgccatcattgcgataaaggaaaggccatcgttgaagatgcctctgccgacagtggtcccaaagatggacccccacccacgaggagcatcgtggaaaaagaagacgttccaaccacgtcttcaaagcaagtggattgatgtgataacatggtggagcacgacacacttgtctactccaaaaatatcaaagatacagtctcagaagaccaaagggcaattgagacttttcaacaaagggtaatatccggaaacctcctcggattccattgcccagctatctgtcactttattgtgaagatagtggaaaaggaaggtggctcctacaaatgccatcattgcgataaaggaaaggccatcgttgaagatgcctctgccgacagtggtcccaaagatggacccccacccacgaggagcatcgtggaaaaagaagacgttccaaccacgtcttcaaagcaagtggattgatgtgatatctccactgacgtaagggatgacgcacaatcccactatccttcgcaagacccttcctctatataaggaagttcatttcatttggagaggacctcgaaattctcaacacaacatatacaaaacaaacgaatctcaagcaatcaagcattctacttctattgcagcaatttaaatcatttcttttaaagcaaaagcaattttctgaaaattttcaccatttacgaacgatagggatccagcgctgagctcgtccgcaaaaatcaccagtctctctctacaaatctatctctctctatttttctccagaataatgtgtgagtagttcccagataagggaattagggttcttatagggtttcgctcatgtgttgagcatataagaaacccttagtatgtatttgtatttgtaaaatacttctatcaataaaatttctaattcctaaaaccaaaatccagtgactataattagccttcctcataagttgcactacttcagcgtcccaattgcacccttaccacgaagacaggtttgtccaatcccatattgcgaccttggcagggggttcgcaagtcccacccgaaacgttgctgaaggctcaggtttctgagcgacaaatgctttaaacgcgagttcccgctcataacctggaccgaatgcgggtcgaccccgggactagtctcgagcacgtggaattcactggccgtcgttttacaacgtcgtgactgggaaaaccctggcgttacccaacttaatcgccttgcagcacatccccctttcgccagctggcgtaatagcgaagaggcccgcaccgatcgcccttcccaacagttgcgcagcctgaatggcgcccgctcctttcgctttcttcccttcctttctcgccacgttcgccggctttccccgtcaagctctaaatcgggggctccctttagggttccgatttagtgctttacggcacctcgaccccaaaaaacttgatttgggtgatggttcacgtagtgggccatcgccctgatagacggtttttcgccctttgacgttggagtccacgttctttaatagtggactcttgttccaaactggaacaacactcaaccctatctcgggctattcttttgatttataagggattttgccgatttcggaaccaccatcaaacaggattttcgcctgctggggcaaaccagcgtggaccgcttgctgcaactctctcagggccaggcggtgaagggcaatcagctgttgcccgtctcactggtgaaaagaaaaaccaccccagtacattaaaaacgtccgcaatgtgttattaagttgtctaagcgtcaatttgtttacaccacaatatatcctgccaccagccagccaacagctccccgaccggcagctcggcacaaaatcaccactcgatacaggcagcccatcagtccgggacggcgtcagcgggagagccgttgtaaggcggcagactttgctcatgttaccgatgctattcggaagaacggcaactaagctgccgggtttgaaacacggatgatctcgcggagggtagcatgttgattgtaacgatgacagagcgttgctgcctgtgatcaaatatcatctccctcgcagagatccgaattatcagccttcttattcatttctcgcttaaccgtgacaggctgtcgatcttgagaactatgccgacataataggaaatcgctggataaagccgctgaggaagctgagtggcgctatttctttagaagtgaacgttgacgatatcaactcccctatccattgctcaccgaatggtacaggtcggggacccgaagttccgactgtcggcctgatgcatccccggctgatcgaccccagatctggggctgagaaagcccagtaaggaaacaactgtaggttcgagtcgcgagatcccccggaaccaaaggaagtaggttaaacccgctccgatcaggccgagccacgccaggccgagaacattggttcctgtaggcatcgggattggcggatcaaacactaaagctactggaacgagcagaagtcctccggccgccagttgccaggcggtaaaggtgagcagaggcacgggaggttgccacttgcgggtcagcacggttccgaacgccatggaaaccgcccccgccaggcccgctgcgacgccgacaggatctagcgctgcgtttggtgtcaacaccaacagcgccacgcccgcagttccgcaaatagcccccaggaccgccatcaatcgtatcgggctacctagcagagcggcagagatgaacacgaccatcagcggctgcacagcgcctaccgtcgccgcgaccccgcccggcaggcggtagaccgaaataaacaacaagctccagaatagcgaaatattaagtgcgccgaggatgaagatgcgcatccaccagattcccgttggaatctgtcggacgatcatcacgagcaataaacccgccggcaacgcccgcagcagcataccggcgacccctcggcctcgctgttcgggctccacgaaaacgccggacagatgcgccttgtgagcgtccttggggccgtcctcctgtttgaagaccgacagcccaatgatctcgccgtcgatgtaggcgccgaatgccacggcatctcgcaaccgttcagcgaacgcctccatgggctttttctcctcgtgctcgtaaacggacccgaacatctctggagctttcttcagggccgacaatcggatctcgcggaaatcctgcacgtcggccgctccaagccgtcgaatctgagccttaatcacaattgtcaattttaatcctctgtttatcggcagttcgtagagcgcgccgtgcgtcccgagcgatactgagcgaagcaagtgcgtcgagcagtgcccgcttgttcctgaaatgccagtaaagcgctggctgctgaacccccagccggaactgaccccacaaggccctagcgtttgcaatgcaccaggtcatcattgacccaggcgtgttccaccaggccgctgcctcgcaactcttcgcaggcttcgccgacctgctcgcgccacttcttcacgcgggtggaatccgatccgcacatgaggcggaaggtttccagcttgagcgggtacggctcccggtgcgagctgaaatagtcgaacatccgtcgggccgtcggcgacagcttgcggtacttctcccatatgaatttcgtgtagtggtcgccagcaaacagcacgacgatttcctcgtcgatcaggacctggcaacgggacgttttcttgccacggtccaggacgcggaagcggtgcagcagcgacaccgattccaggtgcccaacgcggtcggacgtgaagcccatcgccgtcgcctgtaggcgcgacaggcattcctcggccttcgtgtaataccggccattgatcgaccagcccaggtcctggcaaagctcgtagaacgtgaaggtgatcggctcgccgataggggtgcgcttcgcgtactccaacacctgctgccacaccagttcgtcatcgtcggcccgcagctcgacgccggtgtaggtgatcttcacgtccttgttgacgtggaaaatgaccttgttttgcagcgcctcgcgcgggattttcttgttgcgcgtggtgaacagggcagagcgggccgtgtcgtttggcatcgctcgcatcgtgtccggccacggcgcaatatcgaacaaggaaagctgcatttccttgatctgctgcttcgtgtgtttcagcaacgcggcctgcttggcctcgctgacctgttttgccaggtcctcgccggcggtttttcgcttcttggtcgtcatagttcctcgcgtgtcgatggtcatcgacttcgccaaacctgccgcctcctgttcgagacgacgcgaacgctccacggcggccgatggcgcgggcagggcagggggagccagttgcacgctgtcgcgctcgatcttggccgtagcttgctggaccatcgagccgacggactggaaggtttcgcggggcgcacgcatgacggtgcggcttgcgatggtttcggcatcctcggcggaaaaccccgcgtcgatcagttcttgcctgtatgccttccggtcaaacgtccgattcattcaccctccttgcgggattgccccgactcacgccggggcaatgtgcccttattcctgatttgacccgcctggtgccttggtgtccagataatccaccttatcggcaatgaagtcggtcccgtagaccgtctggccgtccttctcgtacttggtattccgaatcttgccctgcacgaataccagcgaccccttgcccaaatacttgccgtgggcctcggcctgagagccaaaacacttgatgcggaagaagtcggtgcgctcctgcttgtcgccggcatcgttgcgccacatctaggtactaaaacaattcatccagtaaaatataatattttattttctcccaatcaggcttgatccccagtaagtcaaaaaatagctcgacatactgttcttccccgatatcctccctgatcgaccggacgcagaaggcaatgtcataccacttgtccgccctgccgcttctcccaagatcaataaagccacttactttgccatctttcacaaagatgttgctgtctcccaggtcgccgtgggaaaagacaagttcctcttcgggcttttccgtctttaaaaaatcatacagctcgcgcggatctttaaatggagtgtcttcttcccagttttcgcaatccacatcggccagatcgttattcagtaagtaatccaattcggctaagcggctgtctaagctattcgtatagggacaatccgatatgtcgatggagtgaaagagcctgatgcactccgcatacagctcgataatcttttcagggctttgttcatcttcatactcttccgagcaaaggacgccatcggcctcactcatgagcagattgctccagccatcatgccgttcaaagtgcaggacctttggaacaggcagctttccttccagccatagcatcatgtccttttcccgttccacatcataggtggtccctttataccggctgtccgtcatttttaaatataggttttcattttctcccaccagcttatataccttagcaggagacattccttccgtatcttttacgcagcggtatttttcgatcagttttttcaattccggtgatattctcattttagccatttattatttccttcctcttttctacagtatttaaagataccccaagaagctaattataacaagacgaactccaattcactgttccttgcattctaaaaccttaaataccagaaaacagctttttcaaagttgttttcaaagttggcgtataacatagtatcgacggagccgattttgaaaccacaattatgggtgatgctgccaacttactgatttagtgtatgatggtgtttttgaggtgctccagtggcttctgtgtctatcagctgtccctcctgttcagctactgacggggtggtgcgtaacggcaaaagcaccgccggacatcagcgctatctctgctctcactgccgtaaaacatggcaactgcagttcacttacaccgcttctcaacccggtacgcaccagaaaatcattgatatggccatgaatggcgttggatgccgggcaacagcccgcattatgggcgttggcctcaacacgattttacgtcacttaaaaaactcaggccgcagtcggtaacctcgcgcatacagccgggcagtgacgtcatcgtctgcgcggaaatggacgaacagtggggctatgtcggggctaaatcgcgccagcgctggctgttttacgcgtatgacagtctccggaagacggttgttgcgcacgtattcggtgaacgcactatggcgacgctggggcgtcttatgagcctgctgtcaccctttgacgtggtgatatggatgacggatggctggccgctgtatgaatcccgcctgaagggaaagctgcacgtaatcagcaagcgatatacgcagcgaattgagcggcataacctgaatctgaggcagcacctggcacggctgggacggaagtcgctgtcgttctcaaaatcggtggagctgcatgacaaagtcatcgggcattatctgaacataaaacactatcaataagttggagtcattacccaattatgatagaatttacaagctataaggttattgtcctgggtttcaagcattagtccatgcaagtttttatgctttgcccattctatagatatattgataagcgcgctgcctatgccttgccccctgaaatccttacatacggcgatatcttctatataaaagatatattatcttatcagtattgtcaatatattcaaggcaatctgcctcctcatcctcttcatcctcttcgtcttggtagctttttaaatatggcgcttcatagagtaattctgtaaaggtccaattctcgttttcatacctcggtataatcttacctatcacctcaaatggttcgctgggtttatcgcacccccgaacacgagcacggcacccgcgaccactatgccaagaatgcccaaggtaaaaattgccggccccgccatgaagtccgtgaatgccccgacggccgaagtgaagggcaggccgccacccaggccgccgccctcactgcccggcacctggtcgctgaatgtcgatgccagcacctgcggcacgtcaatgcttccgggcgtcgcgctcgggctgatcgcccatcccgttactgccccgatcccggcaatggcaaggactgccagcgctgccatttttggggtgaggccgttcgcggccgaggggcgcagcccctggggggatgggaggcccgcgttagcgggccgggagggttcgagaagggggggcaccccccttcggcgtgcgcggtcacgcgcacagggcgcagccctggttaaaaacaaggtttataaatattggtttaaaagcaggttaaaagacaggttagcggtggccgaaaaacgggcggaaacccttgcaaatgctggattttctgcctgtggacagcccctcaaatgtcaataggtgcgcccctcatctgtcagcactctgcccctcaagtgtcaaggatcgcgcccctcatctgtcagtagtcgcgcccctcaagtgtcaataccgcagggcacttatccccaggcttgtccacatcatctgtgggaaactcgcgtaaaatcaggcgttttcgccgatttgcgaggctggccagctccacgtcgccggccgaaatcgagcctgcccctcatctgtcaacgccgcgccgggtgagtcggcccctcaagtgtcaacgtccgcccctcatctgtcagtgagggccaagttttccgcgaggtatccacaacgccggcggccgcggtgtctcgcacacggcttcgacggcgtttctggcgcgtttgcagggccatagacggccgccagcccagcggcgagggcaaccagcccggtgagcgtcgcaaaggcgctcggtcttgccttgctcgtcggtgatgtacttcaccagctccgcgaagtcgctcttcttgatggagcgcatggggacgtgcttggcaatcacgcgcaccccccggccgttttagcggctaaaaaagtcatggctctgccctcgggcggaccacgcccatcatgaccttgccaagctcgtcctgcttctcttcgatcttcgccagcagggcgaggatcgtggcatcaccgaaccgcgccgtgcgcgggtcgtcggtgagccagagtttcagcaggccgcccaggcggcccaggtcgccattgatgcgggccagctcgcggacgtgctcatagtccacgacgcccgtgattttgtagccctggccgacggccagcaggtaggccgacaggctcatgccggccgccgccgccttttcctcaatcgctcttcgttcgtctggaaggcagtacaccttgataggtgggctgcccttcctggttggcttggtttcatcagccatccgcttgccctcatctgttacgccggcggtagccggccagcctcgcagagcaggattcccgttgagcaccgccaggtgcgaataagggacagtgaagaaggaacacccgctcgcgggtgggcctacttcacctatcctgcccggctgacgccgttggatacaccaaggaaagtctacacgaaccctttggcaaaatcctgtatatcgtgcgaaaaaggatggatataccgaaaaaatcgctataatgaccccgaagcagggttatgcagcggaaaagcgccacgcttcccgaagggagaaaggcggacaggtatccggtaagcggcagggtcggaacaggagagcgcacgagggagcttccagggggaaacgcctggtatctttatagtcctgtcgggtttcgccacctctgacttgagcgtcgatttttgtgatgctcgtcaggggggcggagcctatggaaaaacgccagcaacgcggcctttttacggttcctggccttttgctggccttttgctcacatgttctttcctgcgttatcccctgattctgtggataaccgtattaccgcctttgagtgagctgataccgctcgccgcagccgaacgaccgagcgcagcgagtcagtgagcgaggaagcggaagagcgccagaaggccgccagagaggccgagcgcggccgtgaggcttggacgctagggcagggcatgaaaaagcccgtagcgggctgctacgggcgtctgacgcggtggaaagggggaggggatgttgtctacatggctctgctgtagtgagtgggttgcgctccggcagcggtcctgatcaatcgtcaccctttctcggtccttcaacgttcctgacaacgagcctccttttcgccaatccatcgacaatcaccgcgagtccctgctcgaacgctgcgtccggaccggcttcgtcgaaggcgtctatcgcggcccgcaacagcggcgagagcggagcctgttcaacggtgccgccgcgctcgccggcatcgctgtcgccggcctgctcctcaagcacggccccaacagtgaagtagctgattgtcatcagcgcattgacggcgtccccggccgaaaaacccgcctcgcagaggaagcgaagctgcgcgtcggccgtttccatctgcggtgcgcccggtcgcgtgccggcatggatgcgcgcgccatcgcggtaggcgagcagcgcctgcctgaagctgcgggcattcccgatcagaaatgagcgccagtcgtcgtcggctctcggcaccgaatgcgtatgattctccgccagcatggcttcggccagtgcgtcgagcagcgcccgcttgttcctgaagtgccagtaaagcgccggctgctgaacccccaaccgttccgccagtttgcgtgtcgtcagaccgtctacgccgacctcgttcaacaggtccagggcggcacggatcactgtattcggctgcaactttgtcatgcttgacactttatcactgataaacataatatgtccaccaacttatcagtgataaagaatccgcgcgttcaatcggaccagcggaggctggtccggaggccagacgtgaaacccaacatacccctgatcgtaattctgagcactgtcgcgctcgacgctgtcggcatcggcctgattatgccggtgctgccgggcctcctgcgcgatctggttcactcgaacgacgtcaccgcccactatggcattctgctggcgctgtatgcgttggtgcaatttgcctgcgcacctgtgctgggcgcgctgtcggatcgtttcgggcggcggccaatcttgctcgtctcgctggccggcgccagatctggggaaccctgtggttggcatgcacatacaaatggacgaacggataaaccttttcacgcccttttaaatatccgattattctaataaacgctcttttctcttag

SEQ ID NO: 21 - DNA, 18191 bp, Artificial
  V2k_GE_Q2
gtttacccgccaatatatcctgtcaaacactgatagtttaaactgaaggcgggaaacgacaatctgatcatgagcggagaattaagggagtcacgttatgacccccgccgatgacgcgggacaagccgttttacgtttggaactgacagaaccgcaacgttgaaggagccactcagccgcgggtttctggagtttaatgagctaagcacatacgtcagaaaccattattgcgcgttcaaaagtcgcctaaggtcactatcagctagcaaatatttcttgtcaaaaatgctccactgacgttccataaattcccctcggtatccaattagagtctcatattcactctcaatccaaataatctgcaccggatctggatcgtttcgcatgattgaacaagatggattgcacgcaggttctccggccgcttgggtggagaggctattcggctatgactgggcacaacagacaatcggctgctctgatgccgccgtgttccggctgtcagcgcaggggcgcccggttctttttgtcaagaccgacctgtccggtgccctgaatgaactgcaggacgaggcagcgcggctatcgtggctggccacgacgggcgttccttgcgcagctgtgctcgacgttgtcactgaagcgggaagggactggctgctattgggcgaagtgccggggcaggatctcctgtcatctcaccttgctcctgccgagaaagtatccatcatggctgatgcaatgcggcggctgcatacgcttgatccggctacctgcccattcgaccaccaagcgaaacatcgcatcgagcgagcacgtactcggatggaagccggtcttgtcgatcaggatgatctggacgaagagcatcaggggctcgcgccagccgaactgttcgccaggctcaaggcgcgcatgcccgacggcgatgatctcgtcgtgacccatggcgatgcctgcttgccgaatatcatggtggaaaatggccgcttttctggattcatcgactgtggccggctgggtgtggcggaccgctatcaggacatagcgttggctacccgtgatattgctgaagagcttggcggcgaatgggctgaccgcttcctcgtgctttacggtatcgccgctcccgattcgcagcgcatcgccttctatcgccttcttgacgagttcttctgagcgggactctggggttcgaaatgaccgaccaagcgacgcccaacctgccatcacgagatttcgattccaccgccgccttctatgaaaggttgggcttcggaatcgttttccgggacgccggctggatgatcctccagcgcggggatctcatgctggagttcttcgcccacgggatctctgcggaacaggcggtcgaaggtgccgatatcattacgacagcaacggccgacaagcacaacgccacgatcctgagcgacaatatgatcgggcccggcgtccacatcaacggcgtcggcggcgactgcccaggcaagaccgagatgcaccgcgatatcttgctgcgttcggatattttcgtggagttcccgccacagacccggatgatccccgatcgttcaaacatttggcaataaagtttcttaagattgaatcctgttgccggtcttgcgatgattatcatataatttctgttgaattacgttaagcatgtaataattaacatgtaatgcatgacgttatttatgagatgggtttttatgattagagtcccgcaattatacatttaatacgcgatagaaaacaaaatatagcgcgcaaactaggataaattatcgcgcgcggtgtcatctatgttactagatcgggcctcctgtcaatgctggcggcggctctggtggtggttctggtggcggctctgagggtggtggctctgagggtggcggttctgagggtggcggctctgagggaggcggttccggtggtggctctggttccggtgattttgattatgaaaagatggcaaacgctaataagggggctatgaccgaaaatgccgatgaaaacgcgctacagtctgacgctaaaggcaaacttgattctgtcgctactgattacggtgctgctatcgatggtttcattggtgacgtttccggccttgctaatggtaatggtgctactggtgattttgctggctctaattcccaaatggctcaagtcggtgacggtgataattcacctttaatgaataatttccgtcaatatttaccttccctccctcaatcggttgaatgtcgcccttttgtctttggcccaatacgcaaaccgcctctccccgcgcgttggccgattcattaatgcagctggcacgacaggtttcccgactggaaagcgggcagtgagcgcaacgcaattaatgtgagttagctcactcattaggcaccccaggctttacactttatgcttccggctcgtatgttgtgtggaattgtgagcggataacaatttcacacaggaaacagctatgaccatgattacgccaagcttcacgtgaacatggtggagcacgacacacttgtctactccaaaaatatcaaagatacagtctcagaagaccaaagggcaattgagacttttcaacaaagggtaatatccggaaacctcctcggattccattgcccagctatctgtcactttattgtgaagatagtggaaaaggaaggtggctcctacaaatgccatcattgcgataaaggaaaggccatcgttgaagatgcctctgccgacagtggtcccaaagatggacccccacccacgaggagcatcgtggaaaaagaagacgttccaaccacgtcttcaaagcaagtggattgatgtgataacatggtggagcacgacacacttgtctactccaaaaatatcaaagatacagtctcagaagaccaaagggcaattgagacttttcaacaaagggtaatatccggaaacctcctcggattccattgcccagctatctgtcactttattgtgaagatagtggaaaaggaaggtggctcctacaaatgccatcattgcgataaaggaaaggccatcgttgaagatgcctctgccgacagtggtcccaaagatggacccccacccacgaggagcatcgtggaaaaagaagacgttccaaccacgtcttcaaagcaagtggattgatgtgatatctccactgacgtaagggatgacgcacaatcccactatccttcgcaagacccttcctctatataaggaagttcatttcatttggagaggacctcgaaattctcaacacaacatatacaaaacaaacgaatctcaagcaatcaagcattctacttctattgcagcaatttaaatcatttcttttaaagcaaaagcaattttctgaaaattttcaccatttacgaacgatagggatccgagacccaagcttgccaccatgccgaagaagaagcgcaaggtggacaagaagtacagcatcggcctggacatcggtaccaacagcgtgggctgggccgtgatcaccgacgagtacaaggtgcccagcaagaagttcaaggtgctgggcaacaccgaccgccacagcatcaagaagaacctgatcggcgccctgctgttcgacagcggcgagaccgccgaggccacccgcctgaagcgcaccgcccgccgccgctacacccgccgcaagaaccgcatctgctacctgcaggagatcttcagcaacgagatggccaaggtggacgacagcttcttccaccgcctggaggagagcttcctggtggaggaggacaagaagcacgagcgccaccccatcttcggcaacatcgtggacgaggtggcctaccacgagaagtaccccaccatctaccacctgcgcaagaagctggtggacagcaccgacaaggccgacctgcgcctgatctacctggccctggcccacatgatcaagttccgcggccacttcctgatcgagggcgacctgaaccccgacaacagcgacgtggacaagctgttcatccagctggtgcagacctacaaccagctgttcgaggagaaccccatcaacgccagcggcgtggacgccaaggccatcctgagcgcccgcctgagcaagagccgccgcctggagaacctgatcgcccagctgcccggcgagaagaagaacggcctgttcggcaacctgatcgccctgagcctgggcctgacccccaacttcaagagcaacttcgacctggccgaggacgccaagctgcagctgagcaaggacacctacgacgacgacctggacaacctgctggcccagatcggcgaccagtacgccgacctgttcctggccgccaagaacctgagcgacgccatcctgctgagcgacatcctgcgcgtgaacaccgagatcaccaaggcccccctgagcgccagcatgatcaagcgctacgacgagcaccaccaggacctgaccctgctgaaggccctggtgcgccagcagctgcccgagaagtacaaggagatcttcttcgaccagagcaagaacggctacgccggctacatcgacggcggcgccagccaggaggagttctacaagttcatcaagcccatcctggagaagatggacggcaccgaggagctgctggtgaagctgaaccgcgaggacctgctgcgcaagcagcgcaccttcgacaacggcagcatcccccaccagatccacctgggcgagctgcacgccatcctgcgccgccaggaggacttctaccccttcctgaaggacaaccgcgagaagatcgagaagatcctgaccttccgcatcccctactacgtgggccccctggcccgcggcaacagccgcttcgcctggatgacccgcaagagcgaggagaccatcaccccctggaacttcgaggaggtggtggacaagggcgccagcgcccagagcttcatcgagcgcatgaccaacttcgacaagaacctgcccaacgagaaggtgctgcccaagcacagcctgctgtacgagtacttcaccgtgtacaacgagctgaccaaggtgaagtacgtgaccgagggcatgcgcaagcccgccttcctgagcggcgagcagaagaaggccatcgtggacctgctgttcaagaccaaccgcaaggtgaccgtgaagcagctgaaggaggactacttcaagaagatcgagtgcttcgacagcgtggagatcagcggcgtggaggaccgcttcaacgccagcctgggcacctaccacgacctgctgaagatcatcaaggacaaggacttcctggacaacgaggagaacgaggacatcctggaggacatcgtgctgaccctgaccctgttcgaggaccgcgagatgatcgaggagcgcctgaagacctacgcccacctgttcgacgacaaggtgatgaagcagctgaagcgccgccgctacaccggctggggccgcctgagccgcaagcttatcaacggcatccgcgacaagcagagcggcaagaccatcctggacttcctgaagagcgacggcttcgccaaccgcaacttcatgcagctgatccacgacgacagcctgaccttcaaggaggacatccagaaggcccaggtgagcggccagggcgacagcctgcacgagcacatcgccaacctggccggcagccccgccatcaagaagggcatcctgcagaccgtgaaggtggtggacgagctggtgaaggtgatgggccgccacaagcccgagaacatcgtgatcgagatggcccgcgagaaccagaccacccagaagggccagaagaacagccgcgagcgcatgaagcgcatcgaggagggcatcaaggagctgggcagccagatcctgaaggagcaccccgtggagaacacccagctgcagaacgagaagctgtacctgtactacctgcagaacggccgcgacatgtacgtggaccaggagctggacatcaaccgcctgagcgactacgacgtggaccacatcgtgccccagagcttcctgaaggacgacagcatcgacaacaaggtgctgacccgcagcgacaagaaccgcggcaagagcgacaacgtgcccagcgaggaggtggtgaagaagatgaagaactactggcgccagctgctgaacgccaagctgatcacccagcgcaagttcgacaacctgaccaaggccgagcgcggcggcctgagcgagctggacaaggccggcttcatcaagcgccagctggtggagacccgccagatcaccaagcacgtggcccagatcctggacagccgcatgaacaccaagtacgacgagaacgacaagctgatccgcgaggtgaaggtgatcaccctgaagagcaagctggtgagcgacttccgcaaggacttccagttctacaaggtgcgcgagatcaacaactaccaccacgcccacgacgcctacctgaacgccgtggtgggcaccgccctgatcaagaagtaccccaagctggagagcgagttcgtgtacggcgactacaaggtgtacgacgtgcgcaagatgatcgccaagagcgagcaggagatcggcaaggccaccgccaagtacttcttctacagcaacatcatgaacttcttcaagaccgagatcaccctggccaacggcgagatccgcaagcgccccctgatcgagaccaacggcgagaccggcgagatcgtgtgggacaagggccgcgacttcgccaccgtgcgcaaggtgctgagcatgccccaggtgaacatcgtgaagaagaccgaggtgcagaccggcggcttcagcaaggagagcatcctgcccaagcgcaacagcgacaagctgatcgcccgcaagaaggactgggaccccaagaagtacggcggcttcgacagccccaccgtggcctacagcgtgctggtggtggccaaggtggagaagggcaagagcaagaagctgaagagcgtgaaggagctgctgggcatcaccatcatggagcgcagcagcttcgagaagaaccccatcgacttcctggaggccaagggctacaaggaggtgaagaaggacctgatcatcaagctgcccaagtacagcctgttcgagctggagaacggccgcaagcgcatgctggccagcgccggcgagctgcagaagggcaacgagctggccctgcccagcaagtacgtgaacttcctgtacctggccagccactacgagaagctgaagggcagccccgaggacaacgagcagaagcagctgttcgtggagcagcacaagcactacctggacgagatcatcgagcagatcagcgagttcagcaagcgcgtgatcctggccgacgccaacctggacaaggtgctgagcgcctacaacaagcaccgcgacaagcccatccgcgagcaggccgagaacatcatccacctgttcaccctgaccaacctgggcgcccccgccgccttcaagtacttcgacaccaccatcgaccgcaagcgctacaccagcaccaaggaggtgctggacgccaccctgatccaccagagcatcaccggtctgtacgagacccgcatcgacctgagccagctgggcggcgacggcggctccggaaagagaccagctgctaccaagaaggctggacaggctaagaagaagaagtaagagctcgtccgcaaaaatcaccagtctctctctacaaatctatctctctctatttttctccagaataatgtgtgagtagttcccagataagggaattagggttcttatagggtttcgctcatgtgttgagcatataagaaacccttagtatgtatttgtatttgtaaaatacttctatcaataaaatttctaattcctaaaaccaaaatccagtgactataattagccttcctcataagttgcactacttcagcgtcccaattgcacccttaccacgaagacaggtttgtccaatcccatattgcgaccttggcagggggttcgcaagtcccacccgaaacgttgctgaaggctcaggtttctgagcgacaaatgctttaaacgcgagttcccgctcataacctggaccgaatgcgggtcgacagaaatctcaaaattccggcagaacaattttgaatctcgatccgtagaaacgagacggtcattgttttagttccaccacgattatatttgaaatttacgtgagtgtgagtgagacttgcataagaaaataaaatctttagttgggaaaaaattcaataatataaatgggcttgagaaggaagcgagggataggcctttttctaaaataggcccatttaagctattaacaatcttcaaaagtaccacagcgcttaggtaaagaaagcagctgagtttatatatggttagagacgaagtagtgattgccaccaagaatacaagaggttttagagctagaaatagcaagttaaaataaggctagtccgttatcaacttgaaaaagtggcaccgagtcggtgcttttttcaaatgacaattaaccaccgtgtattcgttataacatcaggcagtttaagtcgggacaataggagccgcaatacacagtttaccgcatcttgacctaactagaaatctcaaaattccggcagaacaattttgaatctcgatccgtagaaacgagacggtcattgttttagttccaccacgattatatttgaaatttacgtgagtgtgagtgagacttgcataagaaaataaaatctttagttgggaaaaaattcaataatataaatgggcttgagaaggaagcgagggataggcctttttctaaaataggcccatttaagctattaacaatcttcaaaagtaccacagcgcttaggtaaagaaagcagctgagtttatatatggttagagacgaagtagtgattgcaaaggaagacgggatcatagcgttttagagctagaaatagcaagttaaaataaggctagtccgttatcaacttgaaaaagtggcaccgagtcggtgcttttttactagtctcgagcacgtggaattcactggccgtcgttttacaacgtcgtgactgggaaaaccctggcgttacccaacttaatcgccttgcagcacatccccctttcgccagctggcgtaatagcgaagaggcccgcaccgatcgcccttcccaacagttgcgcagcctgaatggcgcccgctcctttcgctttcttcccttcctttctcgccacgttcgccggctttccccgtcaagctctaaatcgggggctccctttagggttccgatttagtgctttacggcacctcgaccccaaaaaacttgatttgggtgatggttcacgtagtgggccatcgccctgatagacggtttttcgccctttgacgttggagtccacgttctttaatagtggactcttgttccaaactggaacaacactcaaccctatctcgggctattcttttgatttataagggattttgccgatttcggaaccaccatcaaacaggattttcgcctgctggggcaaaccagcgtggaccgcttgctgcaactctctcagggccaggcggtgaagggcaatcagctgttgcccgtctcactggtgaaaagaaaaaccaccccagtacattaaaaacgtccgcaatgtgttattaagttgtctaagcgtcaatttgtttacaccacaatatatcctgccaccagccagccaacagctccccgaccggcagctcggcacaaaatcaccactcgatacaggcagcccatcagtccgggacggcgtcagcgggagagccgttgtaaggcggcagactttgctcatgttaccgatgctattcggaagaacggcaactaagctgccgggtttgaaacacggatgatctcgcggagggtagcatgttgattgtaacgatgacagagcgttgctgcctgtgatcaaatatcatctccctcgcagagatccgaattatcagccttcttattcatttctcgcttaaccgtgacaggctgtcgatcttgagaactatgccgacataataggaaatcgctggataaagccgctgaggaagctgagtggcgctatttctttagaagtgaacgttgacgatatcaactcccctatccattgctcaccgaatggtacaggtcggggacccgaagttccgactgtcggcctgatgcatccccggctgatcgaccccagatctggggctgagaaagcccagtaaggaaacaactgtaggttcgagtcgcgagatcccccggaaccaaaggaagtaggttaaacccgctccgatcaggccgagccacgccaggccgagaacattggttcctgtaggcatcgggattggcggatcaaacactaaagctactggaacgagcagaagtcctccggccgccagttgccaggcggtaaaggtgagcagaggcacgggaggttgccacttgcgggtcagcacggttccgaacgccatggaaaccgcccccgccaggcccgctgcgacgccgacaggatctagcgctgcgtttggtgtcaacaccaacagcgccacgcccgcagttccgcaaatagcccccaggaccgccatcaatcgtatcgggctacctagcagagcggcagagatgaacacgaccatcagcggctgcacagcgcctaccgtcgccgcgaccccgcccggcaggcggtagaccgaaataaacaacaagctccagaatagcgaaatattaagtgcgccgaggatgaagatgcgcatccaccagattcccgttggaatctgtcggacgatcatcacgagcaataaacccgccggcaacgcccgcagcagcataccggcgacccctcggcctcgctgttcgggctccacgaaaacgccggacagatgcgccttgtgagcgtccttggggccgtcctcctgtttgaagaccgacagcccaatgatctcgccgtcgatgtaggcgccgaatgccacggcatctcgcaaccgttcagcgaacgcctccatgggctttttctcctcgtgctcgtaaacggacccgaacatctctggagctttcttcagggccgacaatcggatctcgcggaaatcctgcacgtcggccgctccaagccgtcgaatctgagccttaatcacaattgtcaattttaatcctctgtttatcggcagttcgtagagcgcgccgtgcgtcccgagcgatactgagcgaagcaagtgcgtcgagcagtgcccgcttgttcctgaaatgccagtaaagcgctggctgctgaacccccagccggaactgaccccacaaggccctagcgtttgcaatgcaccaggtcatcattgacccaggcgtgttccaccaggccgctgcctcgcaactcttcgcaggcttcgccgacctgctcgcgccacttcttcacgcgggtggaatccgatccgcacatgaggcggaaggtttccagcttgagcgggtacggctcccggtgcgagctgaaatagtcgaacatccgtcgggccgtcggcgacagcttgcggtacttctcccatatgaatttcgtgtagtggtcgccagcaaacagcacgacgatttcctcgtcgatcaggacctggcaacgggacgttttcttgccacggtccaggacgcggaagcggtgcagcagcgacaccgattccaggtgcccaacgcggtcggacgtgaagcccatcgccgtcgcctgtaggcgcgacaggcattcctcggccttcgtgtaataccggccattgatcgaccagcccaggtcctggcaaagctcgtagaacgtgaaggtgatcggctcgccgataggggtgcgcttcgcgtactccaacacctgctgccacaccagttcgtcatcgtcggcccgcagctcgacgccggtgtaggtgatcttcacgtccttgttgacgtggaaaatgaccttgttttgcagcgcctcgcgcgggattttcttgttgcgcgtggtgaacagggcagagcgggccgtgtcgtttggcatcgctcgcatcgtgtccggccacggcgcaatatcgaacaaggaaagctgcatttccttgatctgctgcttcgtgtgtttcagcaacgcggcctgcttggcctcgctgacctgttttgccaggtcctcgccggcggtttttcgcttcttggtcgtcatagttcctcgcgtgtcgatggtcatcgacttcgccaaacctgccgcctcctgttcgagacgacgcgaacgctccacggcggccgatggcgcgggcagggcagggggagccagttgcacgctgtcgcgctcgatcttggccgtagcttgctggaccatcgagccgacggactggaaggtttcgcggggcgcacgcatgacggtgcggcttgcgatggtttcggcatcctcggcggaaaaccccgcgtcgatcagttcttgcctgtatgccttccggtcaaacgtccgattcattcaccctccttgcgggattgccccgactcacgccggggcaatgtgcccttattcctgatttgacccgcctggtgccttggtgtccagataatccaccttatcggcaatgaagtcggtcccgtagaccgtctggccgtccttctcgtacttggtattccgaatcttgccctgcacgaataccagcgaccccttgcccaaatacttgccgtgggcctcggcctgagagccaaaacacttgatgcggaagaagtcggtgcgctcctgcttgtcgccggcatcgttgcgccacatctaggtactaaaacaattcatccagtaaaatataatattttattttctcccaatcaggcttgatccccagtaagtcaaaaaatagctcgacatactgttcttccccgatatcctccctgatcgaccggacgcagaaggcaatgtcataccacttgtccgccctgccgcttctcccaagatcaataaagccacttactttgccatctttcacaaagatgttgctgtctcccaggtcgccgtgggaaaagacaagttcctcttcgggcttttccgtctttaaaaaatcatacagctcgcgcggatctttaaatggagtgtcttcttcccagttttcgcaatccacatcggccagatcgttattcagtaagtaatccaattcggctaagcggctgtctaagctattcgtatagggacaatccgatatgtcgatggagtgaaagagcctgatgcactccgcatacagctcgataatcttttcagggctttgttcatcttcatactcttccgagcaaaggacgccatcggcctcactcatgagcagattgctccagccatcatgccgttcaaagtgcaggacctttggaacaggcagctttccttccagccatagcatcatgtccttttcccgttccacatcataggtggtccctttataccggctgtccgtcatttttaaatataggttttcattttctcccaccagcttatataccttagcaggagacattccttccgtatcttttacgcagcggtatttttcgatcagttttttcaattccggtgatattctcattttagccatttattatttccttcctcttttctacagtatttaaagataccccaagaagctaattataacaagacgaactccaattcactgttccttgcattctaaaaccttaaataccagaaaacagctttttcaaagttgttttcaaagttggcgtataacatagtatcgacggagccgattttgaaaccacaattatgggtgatgctgccaacttactgatttagtgtatgatggtgtttttgaggtgctccagtggcttctgtgtctatcagctgtccctcctgttcagctactgacggggtggtgcgtaacggcaaaagcaccgccggacatcagcgctatctctgctctcactgccgtaaaacatggcaactgcagttcacttacaccgcttctcaacccggtacgcaccagaaaatcattgatatggccatgaatggcgttggatgccgggcaacagcccgcattatgggcgttggcctcaacacgattttacgtcacttaaaaaactcaggccgcagtcggtaacctcgcgcatacagccgggcagtgacgtcatcgtctgcgcggaaatggacgaacagtggggctatgtcggggctaaatcgcgccagcgctggctgttttacgcgtatgacagtctccggaagacggttgttgcgcacgtattcggtgaacgcactatggcgacgctggggcgtcttatgagcctgctgtcaccctttgacgtggtgatatggatgacggatggctggccgctgtatgaatcccgcctgaagggaaagctgcacgtaatcagcaagcgatatacgcagcgaattgagcggcataacctgaatctgaggcagcacctggcacggctgggacggaagtcgctgtcgttctcaaaatcggtggagctgcatgacaaagtcatcgggcattatctgaacataaaacactatcaataagttggagtcattacccaattatgatagaatttacaagctataaggttattgtcctgggtttcaagcattagtccatgcaagtttttatgctttgcccattctatagatatattgataagcgcgctgcctatgccttgccccctgaaatccttacatacggcgatatcttctatataaaagatatattatcttatcagtattgtcaatatattcaaggcaatctgcctcctcatcctcttcatcctcttcgtcttggtagctttttaaatatggcgcttcatagagtaattctgtaaaggtccaattctcgttttcatacctcggtataatcttacctatcacctcaaatggttcgctgggtttatcgcacccccgaacacgagcacggcacccgcgaccactatgccaagaatgcccaaggtaaaaattgccggccccgccatgaagtccgtgaatgccccgacggccgaagtgaagggcaggccgccacccaggccgccgccctcactgcccggcacctggtcgctgaatgtcgatgccagcacctgcggcacgtcaatgcttccgggcgtcgcgctcgggctgatcgcccatcccgttactgccccgatcccggcaatggcaaggactgccagcgctgccatttttggggtgaggccgttcgcggccgaggggcgcagcccctggggggatgggaggcccgcgttagcgggccgggagggttcgagaagggggggcaccccccttcggcgtgcgcggtcacgcgcacagggcgcagccctggttaaaaacaaggtttataaatattggtttaaaagcaggttaaaagacaggttagcggtggccgaaaaacgggcggaaacccttgcaaatgctggattttctgcctgtggacagcccctcaaatgtcaataggtgcgcccctcatctgtcagcactctgcccctcaagtgtcaaggatcgcgcccctcatctgtcagtagtcgcgcccctcaagtgtcaataccgcagggcacttatccccaggcttgtccacatcatctgtgggaaactcgcgtaaaatcaggcgttttcgccgatttgcgaggctggccagctccacgtcgccggccgaaatcgagcctgcccctcatctgtcaacgccgcgccgggtgagtcggcccctcaagtgtcaacgtccgcccctcatctgtcagtgagggccaagttttccgcgaggtatccacaacgccggcggccgcggtgtctcgcacacggcttcgacggcgtttctggcgcgtttgcagggccatagacggccgccagcccagcggcgagggcaaccagcccggtgagcgtcgcaaaggcgctcggtcttgccttgctcgtcggtgatgtacttcaccagctccgcgaagtcgctcttcttgatggagcgcatggggacgtgcttggcaatcacgcgcaccccccggccgttttagcggctaaaaaagtcatggctctgccctcgggcggaccacgcccatcatgaccttgccaagctcgtcctgcttctcttcgatcttcgccagcagggcgaggatcgtggcatcaccgaaccgcgccgtgcgcgggtcgtcggtgagccagagtttcagcaggccgcccaggcggcccaggtcgccattgatgcgggccagctcgcggacgtgctcatagtccacgacgcccgtgattttgtagccctggccgacggccagcaggtaggccgacaggctcatgccggccgccgccgccttttcctcaatcgctcttcgttcgtctggaaggcagtacaccttgataggtgggctgcccttcctggttggcttggtttcatcagccatccgcttgccctcatctgttacgccggcggtagccggccagcctcgcagagcaggattcccgttgagcaccgccaggtgcgaataagggacagtgaagaaggaacacccgctcgcgggtgggcctacttcacctatcctgcccggctgacgccgttggatacaccaaggaaagtctacacgaaccctttggcaaaatcctgtatatcgtgcgaaaaaggatggatataccgaaaaaatcgctataatgaccccgaagcagggttatgcagcggaaaagcgccacgcttcccgaagggagaaaggcggacaggtatccggtaagcggcagggtcggaacaggagagcgcacgagggagcttccagggggaaacgcctggtatctttatagtcctgtcgggtttcgccacctctgacttgagcgtcgatttttgtgatgctcgtcaggggggcggagcctatggaaaaacgccagcaacgcggcctttttacggttcctggccttttgctggccttttgctcacatgttctttcctgcgttatcccctgattctgtggataaccgtattaccgcctttgagtgagctgataccgctcgccgcagccgaacgaccgagcgcagcgagtcagtgagcgaggaagcggaagagcgccagaaggccgccagagaggccgagcgcggccgtgaggcttggacgctagggcagggcatgaaaaagcccgtagcgggctgctacgggcgtctgacgcggtggaaagggggaggggatgttgtctacatggctctgctgtagtgagtgggttgcgctccggcagcggtcctgatcaatcgtcaccctttctcggtccttcaacgttcctgacaacgagcctccttttcgccaatccatcgacaatcaccgcgagtccctgctcgaacgctgcgtccggaccggcttcgtcgaaggcgtctatcgcggcccgcaacagcggcgagagcggagcctgttcaacggtgccgccgcgctcgccggcatcgctgtcgccggcctgctcctcaagcacggccccaacagtgaagtagctgattgtcatcagcgcattgacggcgtccccggccgaaaaacccgcctcgcagaggaagcgaagctgcgcgtcggccgtttccatctgcggtgcgcccggtcgcgtgccggcatggatgcgcgcgccatcgcggtaggcgagcagcgcctgcctgaagctgcgggcattcccgatcagaaatgagcgccagtcgtcgtcggctctcggcaccgaatgcgtatgattctccgccagcatggcttcggccagtgcgtcgagcagcgcccgcttgttcctgaagtgccagtaaagcgccggctgctgaacccccaaccgttccgccagtttgcgtgtcgtcagaccgtctacgccgacctcgttcaacaggtccagggcggcacggatcactgtattcggctgcaactttgtcatgcttgacactttatcactgataaacataatatgtccaccaacttatcagtgataaagaatccgcgcgttcaatcggaccagcggaggctggtccggaggccagacgtgaaacccaacatacccctgatcgtaattctgagcactgtcgcgctcgacgctgtcggcatcggcctgattatgccggtgctgccgggcctcctgcgcgatctggttcactcgaacgacgtcaccgcccactatggcattctgctggcgctgtatgcgttggtgcaatttgcctgcgcacctgtgctgggcgcgctgtcggatcgtttcgggcggcggccaatcttgctcgtctcgctggccggcgccagatctggggaaccctgtggttggcatgcacatacaaatggacgaacggataaaccttttcacgcccttttaaatatccgattattctaataaacgctcttttctcttag

SEQ ID NO: 22 - DNA, 4935 bp, Artificial
  wild type QPT2S gDNA
atgtttagagctattcctttcactgctacagtgcatccttatgcaattacagctccaaggtctctttaagaagaaaaaaagattcttgaaaatcatgtttttttggttatattctgataaagattgggttttttctgagtttgtgattaaattttgtgtgtaaaattgcaggttggtggtgaaaatgtcagcaatagccaccaagaatacaagagtggagtcattagaggtgaaaccaccagcacacccaacttatgatttaaagggagttatgcaacttgcactctctgaagatgctgggaatttaggtttggtcttagcttatatcttttttctttttaatcttattatattgttaaatgggttgcactcaattttattactttagtaaatgctgtaattacctaatatgtggcctaactgtgtatatattttttacccgttagtgcatagaacttaagcaatttatttaattttggagttgctttatgaagtttagctatagttctttttgttataagagggtccccctggttaaaaaaagagtgtggggaaaagcaaaacaccgaatgtgtttccaccctaaaggtttttgtgtagaaaatttcctatttttggagagtccgggttccggttccccccgggggggaaatttttggaaatttttcccaaaaaattttccccgtgtctcaaaagggttttaaaacccacactttcccttttttggggggattgtggggggggggggggatagctctgtcaaaagttatttttttggtttctcgcccggtgtccgttgcctggtttgtggttcgaccaatccgtttgaggtaaaggaacgactccattctaatctgagacatatggttaaagatagagggtactaaccaccccacttacaacctttggtggtaaaagttacattatttaagatcaatagttgtggatattgtcatgtactctatcagtttgtgcttgatgggaaactttgtgtgattaagtttcttggaaatagcaattttttaagcacctggttacctttgtgaatttgagtactcaatttgaaaaagagatgtctatttattcaatgttttcttgggtgaaatgcaggagatgtgacttgtaaggcgacaattcctcttgatatggaatccgatgctcattttctagcaaaggaagacgggatcatagcaggaattgcacttgctgagatgatattcgcggaagttgatccttcattaaaggtattgattttgctattaagttgttccagtaaccggcatatctatttcgaaaaagtttttgataaagggtaatttttaatttcttcatgatcttattatcaggtggagtggtatgtaaatgatggcgataaagttcataaaggcttgaaatttggcaaagtacaaggtaaactaaatgtgataaaatgatgacttgctaatgatttttcagcttattaatctttccttgacttttgtaggaaacgcttacaacattgttatagctgagagggttgttctcaattttatgcaaagaatgagtggaatagctacactaactaaggtgtgtttctcttcatataaatagtttatccttaaaaaaaatatggaaagatattgccatgaatggaaatggttagtgtcattgatgagttggtttcagtatttcaagttaagtgtaggtctgagactgctgaattgttctatgtcgaagaatactgagtttcgtgcagaacatatgtgttgctccatatttagacattcctctatgatataaaatagctattgttgttcgtcaggttgtgcaattggcttgttaggtcattgatccagctcaaagactgttgaactaagagactttctccgtatttgcatttcaatgtattatggttgaaaaactaaagtctccattcttcaatatttcgagtatgatagcttctctgagatgactatttgccactgatgttacttgcttggcgtgtgagtgctattagtatgaccttatttggattatttttttcttcttcttaataacggtggttcccgtttagtttgcgtgcgcctcgactattccactgggtacatgctgccttccatcggcacaggtatcaggtaactctgttaatgaaggcttagggataaaagggcagcccggtgcactaagctctcgctgtgcatggggtccgaggaagggccggaccacaagcttttgttgtcttttggaatttgaatcctggtatcccatagtttacacccacttcattgaccgctaggttgtcccttgggtgctaatgttatttatattttgaaacttcttgtttttcttttatgctgaagatggtcctgaataggctagcattgtggggatccaacttcctgaattcattgttttcatatttctatgagaagtagccttgaccagaaagataagagttcaagtcttggaaacaaatcgtgtgttttcgttataaggctatgcacatccacttttttgagaccttagatggtgccagagtaatatattgaaaactattttgcaatcagtttatgagaaagactcctctgtttaaataaataattccattccgagatgtcaattagcttaatttcttgcctttatagtagtgattagaagggactgagtttttttttttatttgcaggaaatggcagatgctgcacaccctgcttacatcttggagactaggaaaactgctcctggattacgtttggtggataaatgggcggtaaatatttactcaccaaaatcatctacttgtcaaggctatcacatgtatagtttatcttggctgactttctacctggctttaattaaaggtattgatcggtggggggaagaatcacagaatgggcttatttgatatggtaatgataaaagacaatcacatatctgctgctggaggtgtcggcaaagctctaaaatctgtggatcagtatttggagcaaaataaacttcaaataggggttgaggttggcctcatatacctttgaatttaattcttcgatatggttttagatttgtgtccttatcttttaattttatcgtttgcacatttgatatgtttatttggacctgacagttcaattacctattctaccatccgttacgctatacttttttgtcagttttggtcagataaacatctttctagagccattccaatcataaactatttatatttttgaagatataaactttatggctgatgctacttccaatatcctttcactgaagaactaaattattttctgttgaaaacaaatgttagtccaagaaagagatgtttgacctatatgtgtctttcattaagttggtattcgctcctactttggatagttaagaagactatagataaaatttgacaaggtaaaatttaataaatgtgtcagcatcaagattatataaactttatggctgatgctacttccaatatcctttcactgaagaactaaattattttctgttgaaaacaaatgttagtccaagaaagagatgtttgacctatatgtgtctttcattaagttggtattcgctcctactttggatagttaagaagactatagataaaatttgacaaggtaaaatttaataaatgtgtcagcatcaagattattcctttcactgaagaactaaattattttctgttgaaaacaaatgttagtccaagaaagagatgtttgacctatatgtgtctttcattaagttggtattcgctcctactttggatagttaagaagactatagataaaatttgacaaggtaaaatttaataaatgtgtcagcatcaagaatatgctggtaggaacccaaattgtctgatttgcgatccacgaagttacgcaattgtatttggcagtagagctgtggtcctttcataatgtattctatttgtggtattgaacagagttttaaaccttttctcctatccaacaggttgaaaccaggacaattgcagaagtacgagaggttctggactatgcatctcaaacaaagacttcgttgactaggataatgctggacaatatggttgttccattatctaacggagatattgatgtatccatgcttaaggaggctgtagaattgatcaatgggaggtttgatacggaggtaacgcctggtttcattttcattaactatttcacacgtgtcaactatgttgctcggactcttcaaatatgtagcaggatgcgtgtcaaatcctccaaaagtagtgcatttttggaggatctgacaggggtgcggcatcattttaagagaatctgcgcaacatagagtgtcagaatatggaagacttactgagatgcaatgccttgatttttcataaaaatgaagtaacgcctggatttcctgtaatcgtatatcttttggtgacatgctgttgttgttgtaatggtggcaggcttcaggaaatgttacccttgaaacagtacacaagattggacaaactggtgttacctacatttctaggtatgcatttcgctcttgctatttttttccagagatatccatacaagacagcagaagacacaatatataagagatttctcagtgtttgttattagtatagctgggatgcctttctgtttcttttcttttccttcttataataagatggttagtatacttgccttgttcagacaaacgaaaaagatggttactttacttgcgcatgttagaccaaaaatggtctcagtagatagtctatgttatgtaacaattcttttgataggcaaaagtgacaggtttttatccttagtattaggtgcgcgaaggtttgttatgatactaaaaatagagtttaaatctttgcagtggtgccctgacgcattccgtgaaagcacttgacatttccctgaagatcgatacagagctcgcccttgaagttggaaggcgtacaaaacgagcatga

SEQ ID NO: 23 - DNA, 4067 bp, Artificial
  wild type QPT2T gDNA
atgtttagggctcttcctttcactgcaacagtgcatccatatgcaattacagctccaaggtctctttaagaagaaaaaaagattcttgaaaatcatgtttttttggttatattctgataaagattggatttttatgagtttctgattgaattttgtgtgtaaaattgcaggttggtggtgaaaatgtcagcaatagccaccaagaatacaagagtggagtcactagaggtgaagccaccagcacacccaacttatgatttaaagggtgttatgcaacttgcactctctgaagatgctgggaatttaggtctggtcttagcctatattttttatttatcttattatattgtcaaatgggttgcactcaattttattattttagtaaatgctgtaattacctaatatgtggcctaattgtgtgtatatatattttacaccgttagtgcatataacatagaatttaagctctttatttaatttggagttgctttatgaagtttagctatagtttttttttttgggggcgggggagctccaagcttcaattttcttttttaattgcgtagcctcatttacttacaggtaatgtgttcttagtaagtgttacctttagtttaaggaagggggttggggtagaggcggatcccggatttaaattatatgggttcaacctttaaggttcttagtattaaacctattatatttttaaagttatgggttcagattcagtatgtgttgcaattttagtgaatttttacgttcaaattatgctccgtgtcaaaagtattaggttaagatgaacccggtactataacgctacatacgcctctgtgggtgggggtggagggaatagttccgtcaaaaattatttttattggtttctcgcccggtgtctggtacctgctttgtggtccgactaatccggattgaggtaaaggcgactccattctcaggcttgaacctgagacatttggttaaggatggagggtactaaccaccccacttacaacctttggtggtaaaagtcgcattttttaagatccaagagttgaggatattgtcatgcactatatcagtttgtgcttgatgggaaactttgcttaattaagtttcttggaaatagcaattttttaagcacctagttacctttgtgaatttgagtactcaatttgaaaaagatatatctatttattcaatgtttccttgtgtggaatgcaggagatgtgacttgtaaggcgacgattcctgttgacatggaatccgatgctcattttctagcaaaggaagacgggatcatagcaggaattgcacttgctgagatgatattcgcggaagttgatccttcactaaaggtattgattttgcaattaagttgttccagtaaccggcatatctatttcgaagaagttttttataaagggtaatttttaaattgttcatgttcttattatcaggtggagtggtatgtaaatgatggtgataaagttcataaaggcttgaaatttggcaaagtacaaggtaaactaaatgtgataaaatgatgaattgctaatgattttttggcttattaatctttccttgacgtttgtaggaaacgcttacaacattgttatagctgagagggttgttctcaattttatgcaaagaatgagtggaatagctacactaactaaggtgtgtttctcttcatataactagctcatcactaaaaacaatatggaaagatattgccatgaatggaaatggttagtgtcattgacgagttggtttcagtatttcaagttaagtgtaggtcagagactgctgaattgttctatgccgaagaatagaacaatcaaatgatatataatcaatgaaatatgttggtcacgaatgcggtaatgtatgacttaaaatcttgagatggtacttctagtttaaccaatattcttactgatcaaatacttgaaccaatactcaagcttcattatcaagctcatagactgttgaagtaggagactttgtctgaatttgcaattcaatgagaattagccttagcctatggtaaaagttctccatctcaccagaaagtcaagagtgcaagtcttggaaacaaatcctgtgtaatcgttataaggctatgcacatccactcttctgagactttagatggtgccagagccacatattgaaaaccattttgcaatcaaacaacaacaacatacctagtaaaccaacaatgaggtttggggagggtagcgagtacgcagaccttacccctaccctgtgaaggtagataaactattttcgatagaccctattttgcaatcagtctatgagaaaaactcctctgtttaactaaagaattccgttccgagatgtcaatgagtttaaattcttgcctctgtagtagtgattagaagagagggtttttcttttatttgcaggaaatggcagatgctgcacaccctgcttacatcttggagactaggaaaactgctcctggattacgtttggtggataaatgggcggtaaagatttactcaccaaaatcatctacttgtcaagtctatcacatgtatatttatcttggctgactttctacctggctttaattaaaggtattgattggtggtgggaagaatcacagaatgggcttatttgatatggtaatgataaaagacaatcacatatctgctgctggaggtgtcggcaaagctctaaaatctgtggatcagtatttggagcaaaataaacttcaaataggggttgaggttggcctcataacttttaattaaatcctttgatatgtttataaatctgagtcttatcttttagttttattttttgcacctttgatatgtttacttggacctgacagttcaattacctattctaccatcccttatgctttacttttttgtcatttttggtcagataaacatctttctagagatgtttgacctaaatatttctgtctttcattaagttggtatttgcacctactttggatagttaagaagactaattatgtagatactttttttataagtaaggtaaaattttataaatgtgtcagcatcaagaatatgctggtaggaacccaaattgtctgatttgtgatttcctaagttacgctattgtatttggcagtagagttatggtccttttagaatgtgctcaattttgtggtaattattgaacagaggtttaaacgtttttctcctatccaacaggttgaaaccaggacaattgcagaagtacgtgaggttctagaatatgcatctcaaacaaagacttcgttgactaggataatgctggacaatatggttgttccattatctaacggagatattgatgtatccatgcttaaggaggctgtagaattgatcaatgggaggtttgatacggaggtaacgcctggtttcattttcattgtctgcttcacataagtgtcagaatatagaagaactgtgatgcaatgccatttttcataaaaaagaagtaccgcatggatttcctgtaaacgtatatcttttggtgacatgctgttgttgttgtaatggtggggcaggcttcaggaaatgttacccttgaaacagtacacaagattggacaaactggtgttacctacatttctaggtatgcatttcgctcttgctaatttacttcaaaagatatccatagaatacagcagaagacatatagaagagatttctcagtgtttgttactattagtatagctgggacgtctttctgttccttttgttttccttcatataataagatggttagtttaacttgccttgttcagaaaaacgaaaaagatgattagtttacttgcacacaatagaccagaaacggtctcagtagatagtctatgttatgttaataattcatttgataggcaaaagtgacaggtttttatccttagtattaggcgcgcgaaggtttgttatgatactaaaaatatagagtttaaatctttgcagtggtgccctgacgcattctgtgaaagcacttgacatttccctgaagattgatacagagctcgcccttgaagttggaaggcgtacaaaacgagcatga

SEQ ID NO: 24 - DNA, 1056 bp, Artificial
  wild type QPT2S CDS
atgtttagagctattcctttcactgctacagtgcatccttatgcaattacagctccaaggttggtggtgaaaatgtcagcaatagccaccaagaatacaagagtggagtcattagaggtgaaaccaccagcacacccaacttatgatttaaaggaagttatgaaacttgcactctctgaagatgctgggaatttaggagatgtgacttgtaaggcgacaattcctcttgatatggaatccgatgctcattttctagcaaaggaagacgggatcatagcaggaattgcacttgctgagatgatattcgcggaagttgatccttcattaaaggtggagtggtatgtaaatgatggcgataaagttcataaaggcttgaaatttggcaaagtacaaggaaacgcttacaacattgttatagctgagagggttgttctcaattttatgcaaagaatgagtggaatagctacactaactaaggaaatggcagatgctgcacaccctgcttacatcttggagactaggaaaactgctcctggattacgtttggtggataaatgggcggtattgatcggtggggggaagaatcacagaatgggcttatttgatatggtaatgataaaagacaatcacatatctgctgctggaggtgtcggcaaagctctaaaatctgtggatcagtatttggagcaaaataaacttcaaataggggttgaggttgaaaccaggacaattgaagaagtacgtgaggttctagactatgcatctcaaacaaagacttcgttgactaggataatgctggacaatatggttgttccattatctaacggagatattgatgtatccatgcttaaggaggctgtagaattgatcaatgggaggtttgatacggaggcttcaggaaatgttacccttgaaacagtacacaagattggacaaactggtgttacctacatttctagtggtgccctgacgcattccgtgaaagcacttgacatttccctgaagatcgatacagagctcgcccttgaagttggaaggcgtacaaaacgagcatga

SEQ ID NO: 25 - DNA, 1056 bp, Artificial
  wild type QPT2T CDS
atgtttagggctcttcctttcactgcaacagtgcatccatatgcaattacagctccaaggttggtggtgaaaatgtcagcaatagccaccaagaatacaagagtggagtcattagaggtgaagccaccagcacacccaacttatgatttaaagggtgttatgcaacttgcactctctgaagatgctgggaatttaggagatgtgacttgtaaggcgacgattcctgttgatatggaatccgatgctcattttctagcaaaggaagacgggatcatagcagggattgcacttgctgagatgatattcgcggaagttgatccttcactaaaggtggagtggtatgtaaatgatggtgataaagttcataaaggcttgaaatttggcaaagtacaaggaaacgcttacaacattgttatagctgagagggttgttctcaattttatgcaaagaatgagtggaatagctacactaactaaggaaatggcagatgctgcacaccctgcttacatcttggagactaggaaaactgctcctggattacgtttggtggataaatgggcggtattgatcggtggtgggaagaatcacagaatgggcttatttgatatggtaatgataaaagacaatcacatatctgctgctggaggtgtcggcaaagctctaaaatctgtggatcagtatttggagcaaaataaacttcaaataggggttgaggttgaaaccaggacaattgcagaagtacgtgaggttctagaatatgcatctcaaacaaagacttcgttgactaggataatgctggacaatatggttgttccattatctaacggagatattgatgtatccatgcttaaggaggctgtagaattgatcaatgggaggtttgatacggaggcttcaggaaatgttacccttgaaacagtacacaagattggacaaactggtgttacctacatttctagtggtgccctgacgcattctgtgaaagcacttgacatttccctgaagattgatacagagctcgcccttgaagttggaaggcgtacaaaacgagcatga

SEQ ID NO: 26 - protein, 351 aa, Artificial
  wild type QPT2S amino acid sequence
MFRAIPFTATVHPYAITAPRLVVKMSAIATKNTRVESLEVKPPAHPTYDLKEVMKLALSEDAGNLGDVTCKATIPLDMESDAHFLAKEDGIIAGIALAEMIFAEVDPSLKVEWYVNDGDKVHKGLKFGKVQGNAYNIVIAERVVLNFMQRMSGIATLTKEMADAAHPAYILETRKTAPGLRLVDKWAVLIGGGKNHRMGLFDMVMIKDNHISAAGGVGKALKSVDQYLEQNKLQIGVEVETRTIEEVREVLDYASQTKTSLTRIMLDNMVVPLSNGDIDVSMLKEAVELINGRFDTEASGNVTLETVHKIGQTGVTYISSGALTHSVKALDISLKIDTELALEVGRRTKRA

SEQ ID NO: 27 - protein, 351 aa, Artificial
  wild type QPT2T amino acid sequence
MFRALPFTATVHPYAITAPRLVVKMSAIATKNTRVESLEVKPPAHPTYDLKGVMQLALSEDAGNLGDVTCKATIPVDMESDAHFLAKEDGIIAGIALAEMIFAEVDPSLKVEWYVNDGDKVHKGLKFGKVQGNAYNIVIAERVVLNFMQRMSGIATLTKEMADAAHPAYILETRKTAPGLRLVDKWAVLIGGGKNHRMGLFDMVMIKDNHISAAGGVGKALKSVDQYLEQNKLQIGVEVETRTIAEVREVLEYASQTKTSLTRIMLDNMVVPLSNGDIDVSMLKEAVELINGRFDTEASGNVTLETVHKIGQTGVTYISSGALTHSVKALDISLKIDTELALEVGRRTKRA

SEQ ID NO: 28 - DNA, 1057 bp, Artificial
  mutant QPT2S CDS
atgtttagagctattcctttcactgctacagtgcatccttatgcaattacagctccaaggttggtggtgaaaatgtcagcaatagccaccaagaatacaaagagtggagtcattagaggtgaaaccaccagcacacccaacttatgatttaaaggaagttatgaaacttgcactctctgaagatgctgggaatttaggagatgtgacttgtaaggcgacaattcctcttgatatggaatccgatgctcattttctagcaaaggaagacgggatcatagcaggaattgcacttgctgagatgatattcgcggaagttgatccttcattaaaggtggagtggtatgtaaatgatggcgataaagttcataaaggcttgaaatttggcaaagtacaaggaaacgcttacaacattgttatagctgagagggttgttctcaattttatgcaaagaatgagtggaatagctacactaactaaggaaatggcagatgctgcacaccctgcttacatcttggagactaggaaaactgctcctggattacgtttggtggataaatgggcggtattgatcggtggggggaagaatcacagaatgggcttatttgatatggtaatgataaaagacaatcacatatctgctgctggaggtgtcggcaaagctctaaaatctgtggatcagtatttggagcaaaataaacttcaaataggggttgaggttgaaaccaggacaattgaagaagtacgtgaggttctagactatgcatctcaaacaaagacttcgttgactaggataatgctggacaatatggttgttccattatctaacggagatattgatgtatccatgcttaaggaggctgtagaattgatcaatgggaggtttgatacggaggcttcaggaaatgttacccttgaaacagtacacaagattggacaaactggtgttacctacatttctagtggtgccctgacgcattccgtgaaagcacttgacatttccctgaagatcgatacagagctcgcccttgaagttggaaggcgtacaaaacgagcatga

SEQ ID NO: 29 - DNA, 1055 bp, Artificial
  mutant QPT2T CDS
atgtttagggctcttcctttcactgcaacagtgcatccatatgcaattacagctccaaggttggtggtgaaaatgtcagcaatagccaccaagaatacagagtggagtcattagaggtgaagccaccagcacacccaacttatgatttaaagggtgttatgcaacttgcactctctgaagatgctgggaatttaggagatgtgacttgtaaggcgacgattcctgttgatatggaatccgatgctcattttctagcaaaggaagacgggatcatagcagggattgcacttgctgagatgatattcgcggaagttgatccttcactaaaggtggagtggtatgtaaatgatggtgataaagttcataaaggcttgaaatttggcaaagtacaaggaaacgcttacaacattgttatagctgagagggttgttctcaattttatgcaaagaatgagtggaatagctacactaactaaggaaatggcagatgctgcacaccctgcttacatcttggagactaggaaaactgctcctggattacgtttggtggataaatgggcggtattgatcggtggtgggaagaatcacagaatgggcttatttgatatggtaatgataaaagacaatcacatatctgctgctggaggtgtcggcaaagctctaaaatctgtggatcagtatttggagcaaaataaacttcaaataggggttgaggttgaaaccaggacaattgcagaagtacgtgaggttctagaatatgcatctcaaacaaagacttcgttgactaggataatgctggacaatatggttgttccattatctaacggagatattgatgtatccatgcttaaggaggctgtagaattgatcaatgggaggtttgatacggaggcttcaggaaatgttacccttgaaacagtacacaagattggacaaactggtgttacctacatttctagtggtgccctgacgcattctgtgaaagcacttgacatttccctgaagattgatacagagctcgcccttgaagttggaaggcgtacaaaacgagcatga

SEQ ID NO: 30 - protein, 48 aa, Artificial
  mutant QPT2S amino acid sequence
MFRAIPFTATVHPYAITAPRLVVKMSAIATKNTKSGVIRGETTSTPNL

SEQ ID NO: 31 - protein, 37 aa, Artificial
  mutant QPT2T amino acid sequence
MFRALPFTATVHPYAITAPRLVVKMSAIATKNTEWSH

SEQ ID NO: 32 - DNA, 22 bp, Artificial
  primer sequence of R1q_Q2
ggccacatattaggtaattaca